European Patent Application EP 4 682 166 A1, published January 21, 2026. Title: 抗NMI单克隆抗体或其抗原结合片段及其应用. Applicant: 广州恩迈生物科技有限公司. The sequence listing filed with the application follows.

SEQUENCE LISTING (139 sequences)

SEQ ID NO: 1 - DNA, 405 bp, synthetic construct
  source 1..405: mol_type = other DNA
atggagactgggctgcgctggcttctcctggtcgctgtgctcaaaggtgtccagtgtcagtcgttggaggagtccgggggaggcctggtccagcctgagggatccctgacactcacctgcaaagcctctggattcgacttcagtagcaatgcaatgtgctgggtccgccaggctccagggaaggggctggagtggatcgcatgcattagtagtgctagtagtggtagtagtggtagcacttactacgcgagctgggcgaaaggccgattcaccatctccaaaacctcgtcgaccacggtgactctgcaaatgaccagtctgacagccgcggacatggccacctatttctgtgcgagagatggttacgacttgtggggcccaggcaccctggtcaccgtctcctca

SEQ ID NO: 2 - DNA, 348 bp, synthetic construct
  source 1..348: mol_type = other DNA
cagtcgttggaggagtccgggggaggcctggtccagcctgagggatccctgacactcacctgcaaagcctctggattcgacttcagtagcaatgcaatgtgctgggtccgccaggctccagggaaggggctggagtggatcgcatgcattagtagtgctagtagtggtagtagtggtagcacttactacgcgagctgggcgaaaggccgattcaccatctccaaaacctcgtcgaccacggtgactctgcaaatgaccagtctgacagccgcggacatggccacctatttctgtgcgagagatggttacgacttgtggggcccaggcaccctggtcaccgtctcctca

SEQ ID NO: 3 - protein, 135 aa, synthetic construct
METGLRWLLLVAVLKGVQCQSLEESGGGLVQPEGSLTLTCKASGFDFSSNAMCWVRQAPGKGLEWIACISSASSGSSGSTYYASWAKGRFTISKTSSTTVTLQMTSLTAADMATYFCARDGYDLWGPGTLVTVSS

SEQ ID NO: 4 - protein, 116 aa, synthetic construct
QSLEESGGGLVQPEGSLTLTCKASGFDFSSNAMCWVRQAPGKGLEWIACISSASSGSSGSTYYASWAKGRFTISKTSSTTVTLQMTSLTAADMATYFCARDGYDLWGPGTLVTVSS

SEQ ID NO: 5 - protein, 5 aa, synthetic construct
SNAMC

SEQ ID NO: 6 - protein, 21 aa, synthetic construct
CISSASSGSSGSTYYASWAKG

SEQ ID NO: 7 - protein, 5 aa, synthetic construct
DGYDL

SEQ ID NO: 8 - protein, 8 aa, synthetic construct
GFDFSSNA

SEQ ID NO: 9 - protein, 12 aa, synthetic construct
ISSASSGSSGST

SEQ ID NO: 10 - protein, 7 aa, synthetic construct
ARDGYDL

SEQ ID NO: 11 - protein, 7 aa, synthetic construct
GFDFSSN

SEQ ID NO: 12 - protein, 10 aa, synthetic construct
SSASSGSSGS

SEQ ID NO: 13 - protein, 6 aa, synthetic construct
SSNAMC

SEQ ID NO: 14 - protein, 17 aa, synthetic construct
WIACISSASSGSSGSTY

SEQ ID NO: 15 - protein, 6 aa, synthetic construct
ARDGYD

SEQ ID NO: 16 - protein, 10 aa, synthetic construct
GFDFSSNAMC

SEQ ID NO: 17 - protein, 14 aa, synthetic construct
CISSASSGSSGSTY

SEQ ID NO: 18 - DNA, 399 bp, synthetic construct
  source 1..399: mol_type = other DNA
atggacacgagggcccccactcagctgctggggctcctgctgctctggctcccaggtgccacatttgcccaagtgctgacccagactccatcctccgtgtctgcagctgtgggaggcacagtcaccatcagttgtcagtccagtccgagtgtttataataactacttatcctggtttcagcagaaaccagggcagtctcccaagctcctgatctacagggtatccactctggcatctggggtcccatcgcggttcagcggcagtggatctgggacacagttcactctcaccatcagcggcgtgcagtgtgacgatgctgccacttattactgtgcaggcggttatgatagcgctagtgatacatatgttttcggcggagggaccgaggtggtggtcaaa

SEQ ID NO: 19 - DNA, 330 bp, synthetic construct
  source 1..330: mol_type = other DNA
caagtgctgacccagactccatcctccgtgtctgcagctgtgggaggcacagtcaccatcagttgtcagtccagtccgagtgtttataataactacttatcctggtttcagcagaaaccagggcagtctcccaagctcctgatctacagggtatccactctggcatctggggtcccatcgcggttcagcggcagtggatctgggacacagttcactctcaccatcagcggcgtgcagtgtgacgatgctgccacttattactgtgcaggcggttatgatagcgctagtgatacatatgttttcggcggagggaccgaggtggtggtcaaa

SEQ ID NO: 20 - protein, 133 aa, synthetic construct
MDTRAPTQLLGLLLLWLPGATFAQVLTQTPSSVSAAVGGTVTISCQSSPSVYNNYLSWFQQKPGQSPKLLIYRVSTLASGVPSRFSGSGSGTQFTLTISGVQCDDAATYYCAGGYDSASDTYVFGGGTEVVVK

SEQ ID NO: 21 - protein, 110 aa, synthetic construct
QVLTQTPSSVSAAVGGTVTISCQSSPSVYNNYLSWFQQKPGQSPKLLIYRVSTLASGVPSRFSGSGSGTQFTLTISGVQCDDAATYYCAGGYDSASDTYVFGGGTEVVVK

SEQ ID NO: 22 - protein, 12 aa, synthetic construct
QSSPSVYNNYLS

SEQ ID NO: 23 - protein, 7 aa, synthetic construct
RVSTLAS

SEQ ID NO: 24 - protein, 12 aa, synthetic construct
AGGYDSASDTYV

SEQ ID NO: 25 - protein, 7 aa, synthetic construct
PSVYNNY

SEQ ID NO: 26 - protein, 8 aa, synthetic construct
YNNYLSWF

SEQ ID NO: 27 - protein, 10 aa, synthetic construct
LLIYRVSTLA

SEQ ID NO: 28 - protein, 11 aa, synthetic construct
AGGYDSASDTY

SEQ ID NO: 29 - DNA, 429 bp, synthetic construct
  source 1..429: mol_type = other DNA
atggagactgggctgcgctggcttctcctggtcgctgtgctcaaaggtgtccagtgtcagtcgttggaggagtccgggggagacctggtcaagcctggggcatccctgacactcacctgcacagcctctggattctcctttagtagcagctactacatgtgctgggtccgccaggctccagggaaggggctggagtggatcgcatgcatttatgctggtagtagtggtagcacttactacgcgagctgggcgaaaggccgattcaccatctccaaaacctcgtcgaccacggtgactctgcagatgaccagtctgacagccgcggacacggccacttatttctgtgcgagggagtatagctacgatgactatggtgatttctggggttttaacttgtggggcccaggcaccctggtcaccgtctcctca

SEQ ID NO: 30 - DNA, 372 bp, synthetic construct
  source 1..372: mol_type = other DNA
cagtcgttggaggagtccgggggagacctggtcaagcctggggcatccctgacactcacctgcacagcctctggattctcctttagtagcagctactacatgtgctgggtccgccaggctccagggaaggggctggagtggatcgcatgcatttatgctggtagtagtggtagcacttactacgcgagctgggcgaaaggccgattcaccatctccaaaacctcgtcgaccacggtgactctgcagatgaccagtctgacagccgcggacacggccacttatttctgtgcgagggagtatagctacgatgactatggtgatttctggggttttaacttgtggggcccaggcaccctggtcaccgtctcctca

SEQ ID NO: 31 - protein, 143 aa, synthetic construct
METGLRWLLLVAVLKGVQCQSLEESGGDLVKPGASLTLTCTASGFSFSSSYYMCWVRQAPGKGLEWIACIYAGSSGSTYYASWAKGRFTISKTSSTTVTLQMTSLTAADTATYFCAREYSYDDYGDFWGFNLWGPGTLVTVSS

SEQ ID NO: 32 - protein, 124 aa, synthetic construct
QSLEESGGDLVKPGASLTLTCTASGFSFSSSYYMCWVRQAPGKGLEWIACIYAGSSGSTYYASWAKGRFTISKTSSTTVTLQMTSLTAADTATYFCAREYSYDDYGDFWGFNLWGPGTLVTVSS

SEQ ID NO: 33 - protein, 6 aa, synthetic construct
SSYYMC

SEQ ID NO: 34 - protein, 18 aa, synthetic construct
CIYAGSSGSTYYASWAKG

SEQ ID NO: 35 - protein, 15 aa, synthetic construct
EYSYDDYGDFWGFNL

SEQ ID NO: 36 - protein, 9 aa, synthetic construct
GFSFSSSYY

SEQ ID NO: 37 - protein, 9 aa, synthetic construct
IYAGSSGST

SEQ ID NO: 38 - protein, 17 aa, synthetic construct
AREYSYDDYGDFWGFNL

SEQ ID NO: 39 - protein, 8 aa, synthetic construct
GFSFSSSY

SEQ ID NO: 40 - protein, 7 aa, synthetic construct
YAGSSGS

SEQ ID NO: 41 - protein, 7 aa, synthetic construct
SSSYYMC

SEQ ID NO: 42 - protein, 14 aa, synthetic construct
WIACIYAGSSGSTY

SEQ ID NO: 43 - protein, 16 aa, synthetic construct
AREYSYDDYGDFWGFN

SEQ ID NO: 44 - protein, 11 aa, synthetic construct
GFSFSSSYYMC

SEQ ID NO: 45 - protein, 11 aa, synthetic construct
CIYAGSSGSTY

SEQ ID NO: 46 - DNA, 402 bp, synthetic construct
  source 1..402: mol_type = other DNA
atggacacgagggcccccactcagctgctggggctcctgctgctctggctcccaggtgccagatgtgcccttgtgatgacccagactccatcctccgtgtctgcagctgtgggaggcacagtcaccatcaattgccaggccagtcagaacatttacaccaatttagcctggtatcagcagaaaccagggcagcctcccaagctcctgatctatggtgcatccaatctggaatctggggtcccatcgcggttcaaaggcagtggatctgggacagaatacactctcaccatcagcgacctggagtgtgacgatgctgccacttattactgtcaaagttctttgtatagtcgtattgctgaccgggctaatgctttcggcggagggaccgaggtggtggtcaaa

SEQ ID NO: 47 - DNA, 336 bp, synthetic construct
  source 1..336: mol_type = other DNA
gcccttgtgatgacccagactccatcctccgtgtctgcagctgtgggaggcacagtcaccatcaattgccaggccagtcagaacatttacaccaatttagcctggtatcagcagaaaccagggcagcctcccaagctcctgatctatggtgcatccaatctggaatctggggtcccatcgcggttcaaaggcagtggatctgggacagaatacactctcaccatcagcgacctggagtgtgacgatgctgccacttattactgtcaaagttctttgtatagtcgtattgctgaccgggctaatgctttcggcggagggaccgaggtggtggtcaaa

SEQ ID NO: 48 - protein, 134 aa, synthetic construct
MDTRAPTQLLGLLLLWLPGARCALVMTQTPSSVSAAVGGTVTINCQASQNIYTNLAWYQQKPGQPPKLLIYGASNLESGVPSRFKGSGSGTEYTLTISDLECDDAATYYCQSSLYSRIADRANAFGGGTEVVVK

SEQ ID NO: 49 - protein, 112 aa, synthetic construct
ALVMTQTPSSVSAAVGGTVTINCQASQNIYTNLAWYQQKPGQPPKLLIYGASNLESGVPSRFKGSGSGTEYTLTISDLECDDAATYYCQSSLYSRIADRANAFGGGTEVVVK

SEQ ID NO: 50 - protein, 11 aa, synthetic construct
QASQNIYTNLA

SEQ ID NO: 51 - protein, 7 aa, synthetic construct
GASNLES

SEQ ID NO: 52 - protein, 14 aa, synthetic construct
QSSLYSRIADRANA

SEQ ID NO: 53 - protein, 6 aa, synthetic construct
QNIYTN

SEQ ID NO: 54 - protein, 7 aa, synthetic construct
YTNLAWY

SEQ ID NO: 55 - protein, 10 aa, synthetic construct
LLIYGASNLE

SEQ ID NO: 56 - protein, 13 aa, synthetic construct
QSSLYSRIADRAN

SEQ ID NO: 57 - DNA, 387 bp, synthetic construct
  source 1..387: mol_type = other DNA
atggagactgggctgcgctggcttctcctggtcgctgtgctcagaggtgtccagtgtcagtcgctggaggagtccgggggtcgcctggtcacgcctggaggatccctgacactcacctgcacagtctctggaatcgacctcagtagctatacaatgggctgggtccgccaggctccagggaagggacttgaatacatcggaatcattagtggtggtggtaggacatactacgcgagctgggcgaaaggccgattcaccatctccaaaacctcgtcgaccacggtggatctgaaagtgaccagtctgacaaccgaggacacggccacctatttctgtgccagaatatataccttgtggggccaaggcaccctggtcaccgtctcctcg

SEQ ID NO: 58 - DNA, 330 bp, synthetic construct
  source 1..330: mol_type = other DNA
cagtcgctggaggagtccgggggtcgcctggtcacgcctggaggatccctgacactcacctgcacagtctctggaatcgacctcagtagctatacaatgggctgggtccgccaggctccagggaagggacttgaatacatcggaatcattagtggtggtggtaggacatactacgcgagctgggcgaaaggccgattcaccatctccaaaacctcgtcgaccacggtggatctgaaagtgaccagtctgacaaccgaggacacggccacctatttctgtgccagaatatataccttgtggggccaaggcaccctggtcaccgtctcctcg

SEQ ID NO: 59 - protein, 129 aa, synthetic construct
METGLRWLLLVAVLRGVQCQSLEESGGRLVTPGGSLTLTCTVSGIDLSSYTMGWVRQAPGKGLEYIGIISGGGRTYYASWAKGRFTISKTSSTTVDLKVTSLTTEDTATYFCARIYTLWGQGTLVTVSS

SEQ ID NO: 60 - protein, 110 aa, synthetic construct
QSLEESGGRLVTPGGSLTLTCTVSGIDLSSYTMGWVRQAPGKGLEYIGIISGGGRTYYASWAKGRFTISKTSSTTVDLKVTSLTTEDTATYFCARIYTLWGQGTLVTVSS

SEQ ID NO: 61 - protein, 5 aa, synthetic construct
SYTMG

SEQ ID NO: 62 - protein, 16 aa, synthetic construct
IISGGGRTYYASWAKG

SEQ ID NO: 63 - protein, 4 aa, synthetic construct
IYTL

SEQ ID NO: 64 - protein, 8 aa, synthetic construct
GIDLSSYT

SEQ ID NO: 65 - protein, 7 aa, synthetic construct
ISGGGRT

SEQ ID NO: 66 - protein, 6 aa, synthetic construct
ARIYTL

SEQ ID NO: 67 - protein, 7 aa, synthetic construct
GIDLSSY

SEQ ID NO: 68 - protein, 5 aa, synthetic construct
SGGGR

SEQ ID NO: 69 - protein, 6 aa, synthetic construct
SSYTMG

SEQ ID NO: 70 - protein, 12 aa, synthetic construct
YIGIISGGGRTY

SEQ ID NO: 71 - protein, 5 aa, synthetic construct
ARIYT

SEQ ID NO: 72 - protein, 10 aa, synthetic construct
GIDLSSYTMG

SEQ ID NO: 73 - protein, 9 aa, synthetic construct
IISGGGRTY

SEQ ID NO: 74 - DNA, 405 bp, synthetic construct
  source 1..405: mol_type = other DNA
atggacacgagggcccccactcagctgctggggctcctgctgctctggctcccaggtgccacatttgcccaagtgctgacccagactctagcctccgtgtctgcggctgttggaggcacagtcaccatcaattgccagtccagtcagagtgtttataataacgactacctagcctggtttcagcagaaatcagggcagcctcccaagcaactgatccattctgcatccaaactggcatctggggtcccatcgcggttcaaaggcagtggatctgggacacagttcactctcaccatcaacgacgtgcagtgtgacgatgctgccacttactactgtctaggcggttatgattgttatagtgctgattgtaatgttttcggcggagggaccgaggtggtggtcaaa

SEQ ID NO: 75 - DNA, 336 bp, synthetic construct
  source 1..336: mol_type = other DNA
caagtgctgacccagactctagcctccgtgtctgcggctgttggaggcacagtcaccatcaattgccagtccagtcagagtgtttataataacgactacctagcctggtttcagcagaaatcagggcagcctcccaagcaactgatccattctgcatccaaactggcatctggggtcccatcgcggttcaaaggcagtggatctgggacacagttcactctcaccatcaacgacgtgcagtgtgacgatgctgccacttactactgtctaggcggttatgattgttatagtgctgattgtaatgttttcggcggagggaccgaggtggtggtcaaa

SEQ ID NO: 76 - protein, 135 aa, synthetic construct
MDTRAPTQLLGLLLLWLPGATFAQVLTQTLASVSAAVGGTVTINCQSSQSVYNNDYLAWFQQKSGQPPKQLIHSASKLASGVPSRFKGSGSGTQFTLTINDVQCDDAATYYCLGGYDCYSADCNVFGGGTEVVVK

SEQ ID NO: 77 - protein, 112 aa, synthetic construct
QVLTQTLASVSAAVGGTVTINCQSSQSVYNNDYLAWFQQKSGQPPKQLIHSASKLASGVPSRFKGSGSGTQFTLTINDVQCDDAATYYCLGGYDCYSADCNVFGGGTEVVVK

SEQ ID NO: 78 - protein, 13 aa, synthetic construct
QSSQSVYNNDYLA

SEQ ID NO: 79 - protein, 7 aa, synthetic construct
SASKLAS

SEQ ID NO: 80 - protein, 13 aa, synthetic construct
LGGYDCYSADCNV

SEQ ID NO: 81 - protein, 8 aa, synthetic construct
QSVYNNDY

SEQ ID NO: 82 - protein, 9 aa, unidentified
YNNDYLAWF

SEQ ID NO: 83 - protein, 10 aa, synthetic construct
QLIHSASKLA

SEQ ID NO: 84 - protein, 12 aa, synthetic construct
LGGYDCYSADCN

SEQ ID NO: 85 - DNA, 444 bp, synthetic construct
  source 1..444: mol_type = other DNA
atggagactgggctgcgctggcttctcctggtcgctgtgctcaaaggtgtccagtgtcaggagcagctggaggagtccgggggagacctggtcaagcctgagggatccctgacactcacctgcacagcctctggattctccttcagtgccagctactggatatgctgggtccgccaggctccagggaagggcctggagtggatcgcatgcatttatggtggtagtagtggtagcgcttactacgcgagctgggcgaagggccgattcaccatctccaaaacctcgtcgaccacggtgactctgcaaatgaccagtctgacagccgcggacacggccacttatttctgtgcgagagccggttactataattatggtagtgctggtgatatttatcctagttcctttaagttgtggggcccaggcaccctggtcaccgtctcctca

SEQ ID NO: 86 - DNA, 387 bp, synthetic construct
  source 1..387: mol_type = other DNA
caggagcagctggaggagtccgggggagacctggtcaagcctgagggatccctgacactcacctgcacagcctctggattctccttcagtgccagctactggatatgctgggtccgccaggctccagggaagggcctggagtggatcgcatgcatttatggtggtagtagtggtagcgcttactacgcgagctgggcgaagggccgattcaccatctccaaaacctcgtcgaccacggtgactctgcaaatgaccagtctgacagccgcggacacggccacttatttctgtgcgagagccggttactataattatggtagtgctggtgatatttatcctagttcctttaagttgtggggcccaggcaccctggtcaccgtctcctca

SEQ ID NO: 87 - protein, 148 aa, synthetic construct
METGLRWLLLVAVLKGVQCQEQLEESGGDLVKPEGSLTLTCTASGFSFSASYWICWVRQAPGKGLEWIACIYGGSSGSAYYASWAKGRFTISKTSSTTVTLQMTSLTAADTATYFCARAGYYNYGSAGDIYPSSFKLWGPGTLVTVSS

SEQ ID NO: 88 - protein, 129 aa, synthetic construct
QEQLEESGGDLVKPEGSLTLTCTASGFSFSASYWICWVRQAPGKGLEWIACIYGGSSGSAYYASWAKGRFTISKTSSTTVTLQMTSLTAADTATYFCARAGYYNYGSAGDIYPSSFKLWGPGTLVTVSS

SEQ ID NO: 89 - protein, 6 aa, synthetic construct
ASYWIC

SEQ ID NO: 90 - protein, 18 aa, synthetic construct
CIYGGSSGSAYYASWAKG

SEQ ID NO: 91 - protein, 19 aa, synthetic construct
AGYYNYGSAGDIYPSSFKL

SEQ ID NO: 92 - protein, 9 aa, synthetic construct
GFSFSASYW

SEQ ID NO: 93 - protein, 9 aa, synthetic construct
IYGGSSGSA

SEQ ID NO: 94 - protein, 21 aa, synthetic construct
ARAGYYNYGSAGDIYPSSFKL

SEQ ID NO: 95 - protein, 8 aa, synthetic construct
GFSFSASY

SEQ ID NO: 96 - protein, 7 aa, synthetic construct
YGGSSGS

SEQ ID NO: 97 - protein, 7 aa, synthetic construct
SASYWIC

SEQ ID NO: 98 - protein, 14 aa, synthetic construct
WIACIYGGSSGSAY

SEQ ID NO: 99 - protein, 20 aa, synthetic construct
ARAGYYNYGSAGDIYPSSFK

SEQ ID NO: 100 - protein, 11 aa, synthetic construct
GFSFSASYWIC

SEQ ID NO: 101 - protein, 11 aa, synthetic construct
CIYGGSSGSAY

SEQ ID NO: 102 - DNA, 393 bp, synthetic construct
  source 1..393: mol_type = other DNA
atggacacgagggcccccactcagctgctggggctcctactgctctggctcccaggtgccagatgtgacattgtgatgacccagactccagcctccgtggaggcagctgtgggaggcacagtcaccatcaattgccaggccagtcagagcattagcactgcattagcctggtatcagcagaaaccagggcagcctcccaagctcctgatctatactgcatccaaggtggcatctggggtcccatcgcggttcagcggcagtggatctgggacacagttcactctcaccatcagcgacctggagtgtgccgatgctgccacttactactgtcaaaactattattatagtagtagtagtattactttcggcggagggaccgaggtggtggtcaaa

SEQ ID NO: 103 - DNA, 327 bp, synthetic construct
  source 1..327: mol_type = other DNA
gacattgtgatgacccagactccagcctccgtggaggcagctgtgggaggcacagtcaccatcaattgccaggccagtcagagcattagcactgcattagcctggtatcagcagaaaccagggcagcctcccaagctcctgatctatactgcatccaaggtggcatctggggtcccatcgcggttcagcggcagtggatctgggacacagttcactctcaccatcagcgacctggagtgtgccgatgctgccacttactactgtcaaaactattattatagtagtagtagtattactttcggcggagggaccgaggtggtggtcaaa

SEQ ID NO: 104 - protein, 131 aa, synthetic construct
MDTRAPTQLLGLLLLWLPGARCDIVMTQTPASVEAAVGGTVTINCQASQSISTALAWYQQKPGQPPKLLIYTASKVASGVPSRFSGSGSGTQFTLTISDLECADAATYYCQNYYYSSSSITFGGGTEVVVK

SEQ ID NO: 105 - protein, 109 aa, synthetic construct
DIVMTQTPASVEAAVGGTVTINCQASQSISTALAWYQQKPGQPPKLLIYTASKVASGVPSRFSGSGSGTQFTLTISDLECADAATYYCQNYYYSSSSITFGGGTEVVVK

SEQ ID NO: 106 - protein, 11 aa, synthetic construct
QASQSISTALA

SEQ ID NO: 107 - protein, 7 aa, synthetic construct
TASKVAS

SEQ ID NO: 108 - protein, 11 aa, synthetic construct
QNYYYSSSSIT

SEQ ID NO: 109 - protein, 6 aa, synthetic construct
QSISTA

SEQ ID NO: 110 - protein, 7 aa, synthetic construct
STALAWY

SEQ ID NO: 111 - protein, 10 aa, synthetic construct
LLIYTASKVA

SEQ ID NO: 112 - protein, 10 aa, synthetic construct
QNYYYSSSSI

SEQ ID NO: 113 - DNA, 444 bp, synthetic construct
  source 1..444: mol_type = other DNA
atggagactgggctgcgctggcttctcctggtcgctgtgctcaaaggtgtccagtgtcaggagcagctggtggagtccgggggaggcctggtccagcctgagggatccctgacactcacctgcacagcttctggattctccttcagtagtagttattggatatgctgggtccgccaggctccagggaaggggctggagtggatcgcatgcatttatgctggtactagtggtagcacttactacgcgagctgggcgaaaggccgattcaccatctccaaaacctcgtcgaccactgtggatcttcaaatgaacagtctgacagcggcggacacggccacctatttctgtgcgagagccggttactatacttatggtgctggtgtttatatttatcctagttcctttaagttgtggggcccaggcaccctggtcaccgtctcctca

SEQ ID NO: 114 - DNA, 387 bp, synthetic construct
  source 1..387: mol_type = other DNA
caggagcagctggtggagtccgggggaggcctggtccagcctgagggatccctgacactcacctgcacagcttctggattctccttcagtagtagttattggatatgctgggtccgccaggctccagggaaggggctggagtggatcgcatgcatttatgctggtactagtggtagcacttactacgcgagctgggcgaaaggccgattcaccatctccaaaacctcgtcgaccactgtggatcttcaaatgaacagtctgacagcggcggacacggccacctatttctgtgcgagagccggttactatacttatggtgctggtgtttatatttatcctagttcctttaagttgtggggcccaggcaccctggtcaccgtctcctca

SEQ ID NO: 115 - protein, 148 aa, synthetic construct
METGLRWLLLVAVLKGVQCQEQLVESGGGLVQPEGSLTLTCTASGFSFSSSYWICWVRQAPGKGLEWIACIYAGTSGSTYYASWAKGRFTISKTSSTTVDLQMNSLTAADTATYFCARAGYYTYGAGVYIYPSSFKLWGPGTLVTVSS

SEQ ID NO: 116 - protein, 129 aa, synthetic construct
QEQLVESGGGLVQPEGSLTLTCTASGFSFSSSYWICWVRQAPGKGLEWIACIYAGTSGSTYYASWAKGRFTISKTSSTTVDLQMNSLTAADTATYFCARAGYYTYGAGVYIYPSSFKLWGPGTLVTVSS

SEQ ID NO: 117 - protein, 6 aa, synthetic construct
SSYWIC

SEQ ID NO: 118 - protein, 18 aa, synthetic construct
CIYAGTSGSTYYASWAKG

SEQ ID NO: 119 - protein, 19 aa, synthetic construct
AGYYTYGAGVYIYPSSFKL

SEQ ID NO: 120 - protein, 9 aa, synthetic construct
GFSFSSSYW

SEQ ID NO: 121 - protein, 9 aa, synthetic construct
IYAGTSGST

SEQ ID NO: 122 - protein, 21 aa, synthetic construct
ARAGYYTYGAGVYIYPSSFKL

SEQ ID NO: 123 - protein, 7 aa, synthetic construct
YAGTSGS

SEQ ID NO: 124 - protein, 14 aa, synthetic construct
WIACIYAGTSGSTY

SEQ ID NO: 125 - protein, 20 aa, synthetic construct
ARAGYYTYGAGVYIYPSSFK

SEQ ID NO: 126 - protein, 11 aa, synthetic construct
GFSFSSSYWIC

SEQ ID NO: 127 - protein, 11 aa, synthetic construct
CIYAGTSGSTY

SEQ ID NO: 128 - protein, 19 aa, synthetic construct
AGYYTYGAGVYIYPSSFKL

SEQ ID NO: 129 - DNA, 393 bp, synthetic construct
  source 1..393: mol_type = other DNA
atggacacgagggcccccactcagctgctggggctcctactgctctggctcccaggtgccagatgtgatgtcgtgatgacccagactccagcctccgtggaggcagctgtgggaggcacagtcaccatcaagtgccaggccagtgagagcattggcaatgcattagcctggtatcagcagaaaccaggacagcctcccaagctcctgatctattctgcatccaatctggcatctggggtcccatcgcggttcagtggcagtggatctgggacacagttcactctcaccatcagcgacctggagtgtgccgatgctgccacttactactgtcaaagctattattatagtagtagtagtattactttcggcggagggaccgaggtggtggtcaaa

SEQ ID NO: 130 - DNA, 327 bp, synthetic construct
  source 1..327: mol_type = other DNA
gatgtcgtgatgacccagactccagcctccgtggaggcagctgtgggaggcacagtcaccatcaagtgccaggccagtgagagcattggcaatgcattagcctggtatcagcagaaaccaggacagcctcccaagctcctgatctattctgcatccaatctggcatctggggtcccatcgcggttcagtggcagtggatctgggacacagttcactctcaccatcagcgacctggagtgtgccgatgctgccacttactactgtcaaagctattattatagtagtagtagtattactttcggcggagggaccgaggtggtggtcaaa

SEQ ID NO: 131 - protein, 131 aa, synthetic construct
MDTRAPTQLLGLLLLWLPGARCDVVMTQTPASVEAAVGGTVTIKCQASESIGNALAWYQQKPGQPPKLLIYSASNLASGVPSRFSGSGSGTQFTLTISDLECADAATYYCQSYYYSSSSITFGGGTEVVVK

SEQ ID NO: 132 - protein, 109 aa, synthetic construct
DVVMTQTPASVEAAVGGTVTIKCQASESIGNALAWYQQKPGQPPKLLIYSASNLASGVPSRFSGSGSGTQFTLTISDLECADAATYYCQSYYYSSSSITFGGGTEVVVK

SEQ ID NO: 133 - protein, 11 aa, synthetic construct
QASESIGNALA

SEQ ID NO: 134 - protein, 7 aa, synthetic construct
SASNLAS

SEQ ID NO: 135 - protein, 11 aa, synthetic construct
QSYYYSSSSIT

SEQ ID NO: 136 - protein, 6 aa, synthetic construct
ESIGNA

SEQ ID NO: 137 - protein, 7 aa, synthetic construct
GNALAWY

SEQ ID NO: 138 - protein, 10 aa, synthetic construct
LLIYSASNLA

SEQ ID NO: 139 - protein, 10 aa, synthetic construct
QSYYYSSSSI